European Patent Specification EP 3 955 895 B1, published April 3, 2024. Title: Production of Salipro particles. Applicant: Salipro Biotech AB. The sequence listing filed with the application follows.

SEQUENCE LISTING (46 sequences)

SEQ ID NO: 1 - protein, 81 aa, Homo sapiens
SLPCDICKDVVTAAGDMLKDNATEEEILVYLEKTCDWLPKPNMSASCKEIVDSYLPVILDIIKGEMSRPGEVCSALNLCES

SEQ ID NO: 2 - protein, 79 aa, Homo sapiens
GDVCQDCIQMVTDIQTAVRTNSTFVQALVEHVKEECDRLGPGMADICKNYISQYSEIAIQMMMHMQPKEICALVGFCDE

SEQ ID NO: 3 - protein, 80 aa, Homo sapiens
DVYCEVCEFLVKEVTKLIDNNKTEKEILDAFDKMCSKLPKSLSEECQEVVDTYGSSILSILLEEVSPELVCSMLHLCSGT

SEQ ID NO: 4 - protein, 78 aa, Homo sapiens
GFCEVCKKLVGYLDRNLEKNSTKQEILAALEKGCSFLPDPYQKQCDQFVAEYEPVLIEILVEVMDPSFVCLKIGACPS

SEQ ID NO: 5 - protein, 145 aa, Homo sapiens
MATWALLLLAAMLLGNPGLVFSRLSPEYYDLARAHLRDEEKSCPCLAQEGPQGDLLTKTQELGRDYRTCLTIVQKLKKMVDKPTQRSVSNAATRVCRTGRSRWRDVCRNFMRRYQSRVTQGLVAGETAQQICEDLRLCIPSTGPL

SEQ ID NO: 6 - protein, 129 aa, Sus scrofa
PGLAFSGLTPEHSALARAHPCDGEQFCQNLAPEDPQGDQLLQREELGLICESCRKIIQKLEDMVGPQPNEDTVTQAASRVCDKMKILRGVCKKIMRTFLRRISKDILTGKKPQAICVDIKICKEKTGLI

SEQ ID NO: 7 - protein, 77 aa, Entamoeba histolytica
IPVLCPVCTSLVGKLIDLVLGGAVDKVTDYLETLCAKADGLVETLCTKIVSYGIDKLIEKILEGGSAKLICGLIHAC

SEQ ID NO: 8 - protein, 75 aa, Entamoeba dispar
VVCPVCTSLVGKLIDFVIGGAVDKATDYLETLCAKADGVIETVCSKIVSYGIDKLIEKIIEGGSAKLICGLIHAC

SEQ ID NO: 9 - protein, 77 aa, Entamoeba histolytica
GAILCNLCKDTVKLVENLLTVDGAQAVRQYIDNLCGKASGFLGTLCEKILSFGVDELVKLIENHVDPVVVCEKIHAC

SEQ ID NO: 10 - protein, 75 aa, Entamoeba dispar
GLCNLCKDTVNLIENLLTVDGAQAVRQYIDNLCAKADGFLGTLCNKILSFGVDELVKLIENHVDPVVICEKIHAC

SEQ ID NO: 11 - protein, 77 aa, Entamoeba histolytica
GEILCNLCTGLINTLENLLTTKGADKVKDYISSLCNKASGFIATLCTKVLDFGIDKLIQLIEDKVDANAICAKIHAC

SEQ ID NO: 12 - protein, 75 aa, Entamoeba dispar
IVCNLCTGLINTLENLLTTKGADKVKDYIDSLCNKASGFIATLCTKVLDFGVDKLIQLIEDKVDANAICAKIHAC

SEQ ID NO: 13 - protein, 83 aa, Sus scrofa
GLICESCRKIIQKLEDMVGPQPNEDTVTQAASRVCDKMKILRGVCKKIMRTFLRRISKDILTGKKPQAICVDIKICKEKTGLI

SEQ ID NO: 14 - protein, 78 aa, Sus scrofa
GYFCESCRKIIQKLEDMVGPQPNEDTVTQAASQVCDKLKILRGLCKKIMRSFLRRISWDILTGKKPQAICVDIKICKE

SEQ ID NO: 15 - protein, 83 aa, Equus caballus
GIACWSCRKILQKLEDLVGEQPNEATINEAASRVCRNLGLLRGACKKIMRTCLRLISRDILAGKKPQEVCVDIKLCKHKAGLI

SEQ ID NO: 16 - protein, 84 aa, Bos taurus
GLLCGSCQRIIQHLMDKLGDQPDENTVIEAASKVCGKMGPLKGLCKSITKRFLRRIAADITAGKTSRVVCEDIKMCKSKPVGFI

SEQ ID NO: 17 - protein, 81 aa, Fasciola hepatica
EEPHLDISLCESCTNTVNLVKRLLQNSVVETHIRYLVKYLCKGAGSSQDACIKFIQYEVDGAVGYLIQHNATDICHVIRLC

SEQ ID NO: 18 - protein, 83 aa, Homo sapiens
GRDYRTCLTIVQKLKKMVDKPTQTSVSNAATRVCRTGRSRWRDVCRNFMRRYQSRVIQGLVAGETAQQICEDLRLCIPSTGPL

SEQ ID NO: 19 - protein, 83 aa, Naegleria fowleri
SGICNMCQLLVTQVENWVESNDTIMTLEKKLEQVCSVIPGQYSALCTYAVEQYLPIFIHQVEKQFPALTICQDVHLCSSAQAA

SEQ ID NO: 20 - protein, 73 aa, Clonorchis sinensis
CKHCKTLVGRIQDCWQKGRAKSFVEKTLIFLCKLTGHSEEQCTEHAEEFMKHLDDWITGKTPEELCRSLHMCK

SEQ ID NO: 21 - protein, 83 aa, Naegleria fowleri
PSEFCDVCKYAVQQVDQLALQNEAAIQNALLAACQQLGDNQFGKICNTVVLVYGNELVNALVTYENPTRVCSEQLPLCPKNNT

SEQ ID NO: 22 - protein, 88 aa, Caenorhabditis elegans
NPANPLNLKKHHGVFCDVCKALVEGGEKVGDDDLDAWLDVNIGTLCWTMLLPLHHECEEELKKVKKELKKDIENKDSPDKACKDVDLC

SEQ ID NO: 23 - protein, 83 aa, Homo sapiens
SLPCDICKDVVTAAGDMLKDNATEEEILVYLEKTCDWLPKPNMSASCKEIVDSYLPVILDIIKGEMSRPGEVCSALNLCESLQ

SEQ ID NO: 24 - protein, 83 aa, Bos taurus
SLPCDICKDVITAAGNLLKDNATEQEILMYLERTCDWLPKPNMSASCKEIVDSYLPVILDMIKGQMSHPGEVCSALNLCESLQ

SEQ ID NO: 25 - protein, 83 aa, Mus musculus
SLPCDICKTVVTEAGNLLKDNATQEEILHYLEKTCEWIHDSSLSASCKEVVDSYLPVILDMIKGEMSNPGEVCSALNLCQSLQ

SEQ ID NO: 26 - protein, 83 aa, Gallus gallus
SIPCDLCKELVTVVGKVLKDNGTEDEIRSYLEKTCEFLPDQGLASECKEIVDSYLPVIMDMIKEEFDKPEVVCSALSLCQSLQ

SEQ ID NO: 27 - protein, 83 aa, Danio rerio
TVPCDLCKEVLVVVEQLLKDNVTESELLGYLEKACQLIPDEGLANQCKEIVDNYFPVLMGIIQGELDDPGVVCGALGLCVSQQ

SEQ ID NO: 28 - protein, 83 aa, Xenopus laevis
SMPCDFCKEVVTVLGNYLKDNITQDEIKQYLNKVCDFIPDPGLASTCKQEVSDYFTIVLNLLEQELSNPGVLCSSLGLCTSLQ

SEQ ID NO: 29 - protein, 80 aa, Homo sapiens; identical to SEQ ID NO: 3

SEQ ID NO: 30 - protein, 79 aa, Bos taurus
DIYCEVCEFVVKEVAKLIDNNRTEEEILHALDKVCSKLPTSLAEQCQEVVDTYGRSILSILLDEASPELVCSMLHLCSS

SEQ ID NO: 31 - protein, 79 aa, Mus musculus
VILCQTCQFVMNKFSELIVNNATEELLVKGLSNACGVLPDPARTKCQEVVGTFGPSLLDIFIHEVNPSSLCGVIGLCAA

SEQ ID NO: 32 - protein, 80 aa, Gallus gallus
FSVCEICETMVKEVTGLLESNKTEEEIVHEMEVVCYLLPASVKDQCKDFIEVYGQALIDMLLEATNPEAVCVMLKCCAAN

SEQ ID NO: 33 - protein, 79 aa, Xenopus laevis
NVLCEVCELMVSQLEKLLDNNRTRENIKHGLEKVCKLLPSQYTQKCEDMIEEYSDALIELLEQEANPQAICTALGYCSG

SEQ ID NO: 34 - protein, 79 aa, Danio rerio
SPQCAICEYVMKEIENMIQDQTSEAEIVQAVEKVCNILPSTLTAQCKDLIETYGQAIIDLLVQEADPKTVCSFLALCSG

SEQ ID NO: 35 - protein, 81 aa, Homo sapiens
GGFCEVCKKLVGYLDRNLEKNSTKQEILAALEKGCSFLPDPYQKQCDQFVAEYEPVLIEILVEVMDPSFVCLKIGACPSAH

SEQ ID NO: 36 - protein, 81 aa, Bos taurus
GGFCEVCKKLVGYLDRNLEKNSTKEQILAALEKGCSFLPDQYRKQCDQFVTEYEPVLIEILVEVMDPSFVCLKIGACPAAH

SEQ ID NO: 37 - protein, 81 aa, Mus musculus
GGFCEVCKKLVLYLEHNLEKNSTKEEILAALEKGCSFLPDPYQKQCDDFVAEYEPLLLEILVEVMDPGFVCSKIGVCPSAY

SEQ ID NO: 38 - protein, 81 aa, Gallus gallus
GGFCDICKMIVAYADKELEKNATTTEIEALLEKVCHFLPESVSDQCVQFVEQYEPVVVQLLAEMMDPTFVCTKLGVCGAAK

SEQ ID NO: 39 - protein, 81 aa, Danio rerio
GGFCDVCKMAVRYVDGILEQNATQSEIEEAVLKVCSFLPDAVKDECNQLIEQYEPLLVQLLLQTLDPDFVCMKLGACPEAV

SEQ ID NO: 40 - protein, 81 aa, Xenopus laevis
GDYCAVCKMLMRYVDELLEKNATEIRIKAFLGRICNFLPDSMQNECSALVNEYEPLFIQLLLEALDPSFICIKVNLCQNKK

SEQ ID NO: 41 - protein, 79 aa, Homo sapiens; identical to SEQ ID NO: 2

SEQ ID NO: 42 - protein, 79 aa, Bos taurus
GNVCQDCIQLVTDVQEALRTNSTFVEALVDHAKEECDRLGPGMSDMCKNYINQYSEVAIQMVMHMQPKEICVLAGFCDE

SEQ ID NO: 43 - protein, 83 aa, Gallus gallus
EDVCQDCIRLVTDVQEAVRTNATFVKSLVAHAKEECDRLGPGMSDMCKSYISEYSDLAIQMMMHMKDQQPKDICAMVGFCPSV

SEQ ID NO: 44 - protein, 83 aa, Mus musculus
EDVCQDCMKLVSDVQTAVKTNSSFIQGFVDHVKEDCDRLGPGVSDICKNYVDQYSEVCVQMLMHMQDQQPKEICVLAGFCNEV

SEQ ID NO: 45 - protein, 79 aa, Danio rerio
GDVCQDCVTFISDTQDEARVNSSFINTLIAQVENQCELLGPGMSDMCKEYISQYGPLVFQQLMSMQPKDICARAGFCPT

SEQ ID NO: 46 - protein, 79 aa, Xenopus laevis
GDICNDCTKLVSDVQDALRSNSSFSKKLVDHFLQECNLLDPAIAEMCKSYINQYSDIAIQVLLQMQPKQLCGMAGFCDQ